European Patent Specification EP 3 625 352 B1, published January 24, 2024. Title: Verfahren zur fermentativen de novo Synthese von Harzsäuren. Applicant: Jowat SE. The sequence listing filed with the application follows.

SEQUENCE LISTING (18 sequences)

SEQ ID NO: 1 - DNA, 2445 bp, Ginkgo biloba
atgacagcggcagagacacggccggaccagctgccgcaagaagaaaggttcgtaagtcgcctaaatgccgattatcaccctgccgtgtggaaggacgactttattgatagtttaaccagcccgaacagccatgcaacctccaaatcgtctgttgatgaaactatcaataaacgtatccagaccttggtgaaagaaatacaatgcatgtttcagagcatgggcgatggtgaaacgaatccttctgcttacgataccgcgtgggtggcaagaataccgtcgatcgacggcagtggcgcaccgcagtttccccagacacttcagtggattttaaacaatcagctgccggatggtagctggggtgaagaatgcatctttttggcatatgatcgagtgctgaatacgttagcttgcttgcttacgctcaagatctggaacaaaggcgatattcaagttcagaaaggcgtcgagttcgtacgtaaacatatggaggagatgaaagatgaggccgacaatcatcggccttccgggttcgaggtggtatttccggccatgttagatgaagctaagagccttggcctggacctgccataccatctgccttttattagccagatccaccaaaaacggcaaaagaaattacagaaaattccgttaaatgttttacataaccatcagacagcgcttttatactctctcgaggggctgcaggatgttgtcgattggcaggaaattactaatcttcaatcgcgtgatggaagttttctgagcagtccggcttccaccgcttgtgtcttcatgcatacacaaaacaaacgctgtttgcatttcctgaactttgtgttatctaagttcggtgactatgtaccttgtcactacccgttggatctctttgaacgcctgtgggcggttgacacggtagaacgtctcggcatcgataggtattttaaaaaagaaattaaagaaagccttgattatgtgtaccgttactgggacgcagaacgaggagtgggctgggcgcgatgtaacccgattccagatgtcgatgacaccgcaatggggctgcgaatcctacgcctgcatggctataacgtcagctccgacgtcctggagaatttccgggatgaaaagggcgacttcttttgcttcgcgggccagactcagataggggttaccgataatctgaatctgtaccgttgtagtcaggtgtgctttcctggtgaaaaaattatggaagaagcgaagacgtttacgactaaccacctgcaaaacgccctggccaaaaataacgcattcgataagtgggctgtcaagaaggatctgccgggcgaagtagaatacgccattaagtatccctggcatcgctccatgccgcgtctggaagcccgttcctatatcgagcagtttggttcaaatgacgtctggctcggtaaaacagtatacaaaatgctgtatgttagcaacgagaaatatcttgagctggccaaactggatttcaatatggttcaagctttgcaccaaaaggaaacgcaacacattgtgtcatggtggcgcgagtctggctttaatgatctgacgtttactcgtcagcgtccggtagaaatctatttctccgtggcggtgagtatgttcgaaccagagttcgccgcttgtcgcattgcctacgcaaaaacctcatgcctcgcggtgatcctggacgatctgtatgatacgcatggtagtctggatgacctcaaattgtttagcgaggcggtccgccgttgggatattagtgttcttgacagcgtgcgcgataaccaactgaaggtgtgttttctcggactgttcaacacagtgaacggtttcggcaaagatgggctgaaagaacagggccgcgatgtcttgggttatttgcgcaaggtgtgggaaggtttgctagcgtcctacacgaaagaggcggaatggagcgcagcaaagtatgtgccaacctttaatgaatatgtcgagaatgcaaaagtttcaattgcgctcgccaccgtagttctgaattcaatcttctttaccggcgagctgctgccagattacattctccagcaggtagacctgcgctcgaaattcttacatctggtgagtctcaccggccgtttgataaacgataccaaaacataccaggccgaacgtaaccgcggggagctggtttcttcggtccaatgttacatgcgcgagaacccggagtgtactgaagaggaagctctcagccacgtctacggcataattgacaacgcactgaaggaactgaactgggagctagcaaaccctgcgtccaacgcgcccttatgcgtgcgccgtctgttgtttaataccgctcgtgtcatgcagcttttttacatgtatcgtgacggttttggaatttcggataaagaaatgaaagatcacgtgtcccgtaccttatttgacccggtagcatga

SEQ ID NO: 2 - protein, 814 aa, Ginkgo biloba
MTAAETRPDQLPQEERFVSRLNADYHPAVWKDDFIDSLTSPNSHATSKSSVDETINKRIQTLVKEIQCMFQSMGDGETNPSAYDTAWVARIPSIDGSGAPQFPQTLQWILNNQLPDGSWGEECIFLAYDRVLNTLACLLTLKIWNKGDIQVQKGVEFVRKHMEEMKDEADNHRPSGFEVVFPAMLDEAKSLGLDLPYHLPFISQIHQKRQKKLQKIPLNVLHNHQTALLYSLEGLQDVVDWQEITNLQSRDGSFLSSPASTACVFMHTQNKRCLHFLNFVLSKFGDYVPCHYPLDLFERLWAVDTVERLGIDRYFKKEIKESLDYVYRYWDAERGVGWARCNPIPDVDDTAMGLRILRLHGYNVSSDVLENFRDEKGDFFCFAGQTQIGVTDNLNLYRCSQVCFPGEKIMEEAKTFTTNHLQNALAKNNAFDKWAVKKDLPGEVEYAIKYPWHRSMPRLEARSYIEQFGSNDVWLGKTVYKMLYVSNEKYLELAKLDFNMVQALHQKETQHIVSWWRESGFNDLTFTRQRPVEIYFSVAVSMFEPEFAACRIAYAKTSCLAVILDDLYDTHGSLDDLKLFSEAVRRWDISVLDSVRDNQLKVCFLGLFNTVNGFGKDGLKEQGRDVLGYLRKVWEGLLASYTKEAEWSAAKYVPTFNEYVENAKVSIALATVVLNSIFFTGELLPDYILQQVDLRSKFLHLVSLTGRLINDTKTYQAERNRGELVSSVQCYMRENPECTEEEALSHVYGIIDNALKELNWELANPASNAPLCVRRLLFNTARVMQLFYMYRDGFGISDKEMKDHVSRTLFDPVA

SEQ ID NO: 3 - DNA, 939 bp, Pantoea agglomerans
atgcattatccgtttataaggacagcccgaatgacggtctgcgcaaaaaaacacgttcatctcactcgcgatgctgcggagcagttactggctgatattgatcgacgccttgatcagttattgcccgtggagggagaacgggatgttgtgggtgccgcgatgcgtgaaggtgcgctggcaccgggaaaacgtattcgccccatgttgctgttgctgaccgcccgcgatctgggttgcgctgtcagccatgacggattactggatttggcctgtgcggtggaaatggtccacgcggcttcgctgatccttgacgatatgccctgcatggacgatgcgaagctgcggcgcggacgccctaccattcattctcattacggagagcatgtggcaatactggcggcggttgccttgctgagtaaagcctttggcgtaattgccgatgcagatggcctcacgccgctggcaaaaaatcgggcggtttctgaactgtcaaacgccatcggcatgcaaggattggttcagggtcagttcaaggatctgtctgaaggggataagccgcgcagcgctgaagctattttgatgacgaatcactttaaaaccagcacgctgttttgtgcctccatgcagatggcctcgattgttgcgaatgcctccagcgaagcgcgtgattgcctgcatcgtttttcacttgatcttggtcaggcatttcaactgctggacgatttgaccgatggcatgaccgacaccggtaaggatagcaatcaggacgccggtaaatcgacgctggtcaatctgttaggcccgagggcggttgaagaacgtctgagacaacatcttcagcttgccagtgagcatctctctgcggcctgccaacacgggcacgccactcaacattttattcaggcctggtttgacaaaaaactcgctgccgtcagttaa

SEQ ID NO: 4 - protein, 312 aa, Pantoea agglomerans
MHYPFIRTARMTVCAKKHVHLTRDAAEQLLADIDRRLDQLLPVEGERDVVGAAMREGALAPGKRIRPMLLLLTARDLGCAVSHDGLLDLACAVEMVHAASLILDDMPCMDDAKLRRGRPTIHSHYGEHVAILAAVALLSKAFGVIADADGLTPLAKNRAVSELSNAIGMQGLVQGQFKDLSEGDKPRSAEAILMTNHFKTSTLFCASMQMASIVANASSEARDCLHRFSLDLGQAFQLLDDLTDGMTDTGKDSNQDAGKSTLVNLLGPRAVEERLRQHLQLASEHLSAACQHGHATQHFIQAWFDKKLAAVS

SEQ ID NO: 5 - DNA, 1044 bp, Pantoea agglomerans
atgaaggacgagcgccttgttcagcgtaagaacgatcatctggatatcgttctcgacccccgtcgcgccgtaactcaggctagcgcaggttttgagcgctggcgctttacccactgcgccctgccagagctgaattttagcgacatcacgctggaaaccaccttcctgaatcggcagctacaggctccgctgctgatcagctccatgaccggcggcgttgagcgctcgcgccatatcaaccgccacctcgccgaggcggcgcaggtgctaaaaattgcgatgggggtgggctcccagcgcgtcgccattgagagcgacgcgggcttagggctggataaaaccctgcggcagctggctccggacgtgccgctgctggcgaacctcggcgcggcgcagctgaccggcagaaaaggtattgattacgcccgacgggccgtggagatgatcgaggcggatgcgctgattgtgcacctaaacccgctgcaggaggcgctacagcccggcggcgatcgcgactggcgcggacggctggcggctattgaaactctggtccgcgagctgcccgttccgctggtggtgaaagaggtgggagccggtatctcccgaaccgtggccgggcagctgatcgatgccggcgttaccgtgattgacgtcgcgggcgcgggcggcaccagctgggccgccgttgaaggcgagcgggcggccaccgagcagcagcgcagcgtggccaacgtctttgccgactgggggatccccaccgctgaggcgctggttgacattgccgaggcctggccgcagatgccccttattgcctcgggcgggattaaaaacggcgtcgacgcggcgaaagcgctgcggctcggcgcgtgcatggtagggcaggccgccgccgtgctcggcagcgcaggcgtctccacggagaaggtgatcgatcacttcaacgtgattattgagcagctgcgggtggcctgcttctgcaccggcagccgcagcctgagcgatctaaagcaggctgatatccgctatgtgcgtgatacgccataa

SEQ ID NO: 6 - protein, 346 aa, Pantoea agglomerans
MKDERLVQRKNDHLDIVLDPRRAVTQASAGFERWRFTHCALPELNFSDITLETTFLNRQLQAPLLISSMTGGVERSRHINRHLAEAAQVLKIAMGVGSQRVAIESDAGLGLDKTLRQLAPDVPLLANLGAAQLTGRKGIDYARRAVEMIEADALIVHLNPLQEALQPGGDRDWRGRLAAIETLVRELPVPLVVKEVGAGISRTVAGQLIDAGVTVIDVAGAGGTSWAAVEGERAATEQQRSVANVFADWGIPTAEALVDIAEAWPQMPLIASGGIKNGVDAAKALRLGACMVGQAAAVLGSAGVSTEKVIDHFNVIIEQLRVACFCTGSRSLSDLKQADIRYVRDT

SEQ ID NO: 7 - DNA, 1362 bp, Picea sitchensis
atgatacagcggggcccaaagatgagcaacaaagaagtacacttacctccggggagcacgggttggcctttaataggtgaaacgttctcctactaccgttctatgacctcaaatcacccgcgtaagtttattgacgatcgagagaagcgatatgactcagacatcttcatctcgcatctctttggtggtcgtacagttgtttccgcagatccgcaatttaataagtttgtccttcagaatgaaggccgcttcttccaagcgcaatacccgaaggcattaaaggccctaatcggcaactatgggctgctatcagttcacggcgacctacaacgaaaattacacggtattgcagtgaacctgctacgattcgagcgactaaaagtagatttcatggaagaaattcagaacctcgtgcacagtacattagatagatgggctgacatgaaggaaatttcattgcaaaacgaatgtcaccagatggtactgaacctgatggcgaaacagctgctcgatctctcaccaagcaaggagacttccgatatatgcgaactgttcgttgattatacaaacgccgttatagccatccctattaagatacctggctctacgtatgcaaaggggctaaaagccagagagttattaatcaagaagatctccgagatgataaaagagaggaggaaccatcctgaggtggtgcataacgacctcctaactaagctcgttgaagagggcctcatcagcgatgaaatcatttgtgactttatcctcttcctgcttttcgcaggtcatgaaaccagtagtcgcgccatgacattcgcaattaagttcttgacatattgcccaaaagcattaaaacaaatgaaagaggagcacgatgctatccttaaatccaaaggagggcataagaagctgaactgggacgattacaaatccatggcgtttactcagtgcgtgattaatgagacactacggttagggaacttcgggccaggagtctttcgtgaagctaaagaagatactaaagtaaaagactgcttgatccctaagggttgggtggtatttgcctttcttaccgccacgcacctacatgaaaagttccacaatgaagctctgacttttaatccgtggcgttggcaattagacaaagatgttcccgacgattctctcttctcgccctttggcggaggggcccgactgtgccctggtagtcacttggccaagctcgagcttagtctgttccttcacatatttatcacacgcttctcgtgggaggcgcgagcggacgatcggaccagctatttccccttaccctacttaacgaagggtttccctatatctctgcacggacgcgtagaaaatgaa

SEQ ID NO: 8 - protein, 454 aa, Picea sitchensis
MIQRGPKMSNKEVHLPPGSTGWPLIGETFSYYRSMTSNHPRKFIDDREKRYDSDIFISHLFGGRTVVSADPQFNKFVLQNEGRFFQAQYPKALKALIGNYGLLSVHGDLQRKLHGIAVNLLRFERLKVDFMEEIQNLVHSTLDRWADMKEISLQNECHQMVLNLMAKQLLDLSPSKETSDICELFVDYTNAVIAIPIKIPGSTYAKGLKARELLIKKISEMIKERRNHPEVVHNDLLTKLVEEGLISDEIICDFILFLLFAGHETSSRAMTFAIKFLTYCPKALKQMKEEHDAILKSKGGHKKLNWDDYKSMAFTQCVINETLRLGNFGPGVFREAKEDTKVKDCLIPKGWVVFAFLTATHLHEKFHNEALTFNPWRWQLDKDVPDDSLFSPFGGGARLCPGSHLAKLELSLFLHIFITRFSWEARADDRTSYFPLPYLTKGFPISLHGRVENE

SEQ ID NO: 9 - DNA, 1911 bp, Hybrid Zyngiber officinale/Arabidopsis
atggggaggaagcccgccgagccgccgaagccgctggtggtgaagacccagatggatgcggaggaggaggaccaagggaagaagaaggtcaccgtcttcttcgggacgcagaccgggacggctgaggggttcgcgaaggcgctggctgaggaggcaaaggcacggtaccctaatgccatatttaaagtcgtggatatcgacgaatatgctgctgaggatgatgagtacgaggagaacctgaaaaaggagagcttggctttgttcttcttggctacgtatggagatggtgagcctactgataatgctgcccggttctacaaatggtttacagaggggaaagagagaggaatctggttggaaaatcttcaatttggcgtgtttggtttgggcaatcggcaatatgaacattttaataaggttgctgtggtggtcgatgaactgcttcatgagcaaggcgccaagcacattgtccaagtggggttgggagatgatgatcagtgtattgaggatgacttctctgcatggagggagcttctttggccggagttggataagttgcttcaggatgaaaatgagacagctgttgccacaccatacactgcagctgtgttagaatacagagtttctattcacgactctgaagatgccaaattcaatgatataaacatggcaaatgggaatggttacactgtgtttgatgctcaacatccttacaaagcaaatgtcgctgttaaaagggagcttcatactcccgagtctgatcgttcttgtatccatttggaatttgacattgctggaagtggacttacgtatgaaactggagatcatgttggtgtactttgtgataacttaagtgaaactgtagatgaagctcttagattgctggatatgtcacctgatacttatttctcacttcacgctgaaaaagaagacggcacaccaatcagcagctcactgcctcctcccttcccaccttgcaacttgagaacagcgcttacacgatatgcatgtcttttgagttctccaaagaagtctgctttagttgcgttggctgctcatgcatctgatcctaccgaagcagaacgattaaaacaccttgcttcacctgctggaaaggatgaatattcaaagtgggtagtagagagtcaaagaagtctacttgaggtgatggccgagtttccttcagccaagccaccacttggtgtcttcttcgctggagttgctccaaggttgcagcctaggttctattcgatatcatcatcgcccaagattgctgaaactagaattcacgtcacatgtgcactggtttatgagaaaatgccaactggcaggattcataagggagtgtgttccacttggatgaagaatgctgtgccttacgagaagagtgaaaactgttcctcggcgccgatatttgttaggcaatccaacttcaagcttccttctgatcctttagtacctatcatcatgattggacctggcacagggttggcacctttcaggggcttcttacaggaaaggttggcattgaaaaatgatggggtggaacttggtcattctattctcttctttggatgcagaaaccgcaaaatggacttcatttacgaggatgagttgaacaattttgtcaaaacaggcgccctttctgagttgattgtagccttctcccgtgagggtccaactaaacaatatgtgcaacataaaatgactgagaaagcaacggaactttggaatatcatctcccaaggcggatatgtatacgtgtgtggagatgctaagggcatggctagagatgttcacagagttcttcatactattgctcaagagcagggaggtatggatagctccaaaacagaaagcttcatcaagagtttgcaaatggaagggagatacctaagagatgtatggtga

SEQ ID NO: 10 - protein, 636 aa, Hybrid Zyngiber officinale/Arabidopsis
MGRKPAEPPKPLVVKTQMDAEEEDQGKKKVTVFFGTQTGTAEGFAKALAEEAKARYPNAIFKVVDIDEYAAEDDEYEENLKKESLALFFLATYGDGEPTDNAARFYKWFTEGKERGIWLENLQFGVFGLGNRQYEHFNKVAVVVDELLHEQGAKHIVQVGLGDDDQCIEDDFSAWRELLWPELDKLLQDENETAVATPYTAAVLEYRVSIHDSEDAKFNDINMANGNGYTVFDAQHPYKANVAVKRELHTPESDRSCIHLEFDIAGSGLTYETGDHVGVLCDNLSETVDEALRLLDMSPDTYFSLHAEKEDGTPISSSLPPPFPPCNLRTALTRYACLLSSPKKSALVALAAHASDPTEAERLKHLASPAGKDEYSKWVVESQRSLLEVMAEFPSAKPPLGVFFAGVAPRLQPRFYSISSSPKIAETRIHVTCALVYEKMPTGRIHKGVCSTWMKNAVPYEKSENCSSAPIFVRQSNFKLPSDPLVPIIMIGPGTGLAPFRGFLQERLALKNDGVELGHSILFFGCRNRKMDFIYEDELNNFVKTGALSELIVAFSREGPTKQYVQHKMTEKATELWNIISQGGYVYVCGDAKGMARDVHRVLHTIAQEQGGMDSSKTESFIKSLQMEGRYLRDVW

SEQ ID NO: 11 - DNA, 7693 bp, pGT1695
acccagtttcatcattccattttattttgcgagcgagcgcacacttgtgaattatctcaatagcagtgtgaaataacataattgagcaactgaaagggagtgcccaatattacgacatcatccatcacgcggagttacctgattatgacacagagggcccaccatcaccatcaccattccatgatacagcggggcccaaagatgagcaacaaagaagtacacttacctccggggagcacgggttggcctttaataggtgaaacgttctcctactaccgttctatgacctcaaatcacccgcgtaagtttattgacgatcgagagaagcgatatgactcagacatcttcatctcgcatctctttggtggtcgtacagttgtttccgcagatccgcaatttaataagtttgtccttcagaatgaaggccgcttcttccaagcgcaatacccgaaggcattaaaggccctaatcggcaactatgggctgctatcagttcacggcgacctacaacgaaaattacacggtattgcagtgaacctgctacgattcgagcgactaaaagtagatttcatggaagaaattcagaacctcgtgcacagtacattagatagatgggctgacatgaaggaaatttcattgcaaaacgaatgtcaccagatggtactgaacctgatggcgaaacagctgctcgatctctcaccaagcaaggagacttccgatatatgcgaactgttcgttgattatacaaacgccgttatagccatccctattaagatacctggctctacgtatgcaaaggggctaaaagccagagagttattaatcaagaagatctccgagatgataaaagagaggaggaaccatcctgaggtggtgcataacgacctcctaactaagctcgttgaagagggcctcatcagcgatgaaatcatttgtgactttatcctcttcctgcttttcgcaggtcatgaaaccagtagtcgcgccatgacattcgcaattaagttcttgacatattgcccaaaagcattaaaacaaatgaaagaggagcacgatgctatccttaaatccaaaggagggcataagaagctgaactgggacgattacaaatccatggcgtttactcagtgcgtgattaatgagacactacggttagggaacttcgggccaggagtctttcgtgaagctaaagaagatactaaagtaaaagactgcttgatccctaagggttgggtggtatttgcctttcttaccgccacgcacctacatgaaaagttccacaatgaagctctgacttttaatccgtggcgttggcaattagacaaagatgttcccgacgattctctcttctcgccctttggcggaggggcccgactgtgccctggtagtcacttggccaagctcgagcttagtctgttccttcacatatttatcacacgcttctcgtgggaggcgcgagcggacgatcggaccagctatttccccttaccctacttaacgaagggtttccctatatctctgcacggacgcgtagaaaatgaaatgtccggttctgggatggggaggaagcccgccgagccgccgaagccgctggtggtgaagacccagatggatgcggaggaggaggaccaagggaagaagaaggtcaccgtcttcttcgggacgcagaccgggacggctgaggggttcgcgaaggcgctggctgaggaggcaaaggcacggtaccctaatgccatatttaaagtcgtggatatcgacgaatatgctgctgaggatgatgagtacgaggagaacctgaaaaaggagagcttggctttgttcttcttggctacgtatggagatggtgagcctactgataatgctgcccggttctacaaatggtttacagaggggaaagagagaggaatctggttggaaaatcttcaatttggcgtgtttggtttgggcaatcggcaatatgaacattttaataaggttgctgtggtggtcgatgaactgcttcatgagcaaggcgccaagcacattgtccaagtggggttgggagatgatgatcagtgtattgaggatgacttctctgcatggagggagcttctttggccggagttggataagttgcttcaggatgaaaatgagacagctgttgccacaccatacactgcagctgtgttagaatacagagtttctattcacgactctgaagatgccaaattcaatgatataaacatggcaaatgggaatggttacactgtgtttgatgctcaacatccttacaaagcaaatgtcgctgttaaaagggagcttcatactcccgagtctgatcgttcttgtatccatttggaatttgacattgctggaagtggacttacgtatgaaactggagatcatgttggtgtactttgtgataacttaagtgaaactgtagatgaagctcttagattgctggatatgtcacctgatacttatttctcacttcacgctgaaaaagaagacggcacaccaatcagcagctcactgcctcctcccttcccaccttgcaacttgagaacagcgcttacacgatatgcatgtcttttgagttctccaaagaagtctgctttagttgcgttggctgctcatgcatctgatcctaccgaagcagaacgattaaaacaccttgcttcacctgctggaaaggatgaatattcaaagtgggtagtagagagtcaaagaagtctacttgaggtgatggccgagtttccttcagccaagccaccacttggtgtcttcttcgctggagttgctccaaggttgcagcctaggttctattcgatatcatcatcgcccaagattgctgaaactagaattcacgtcacatgtgcactggtttatgagaaaatgccaactggcaggattcataagggagtgtgttccacttggatgaagaatgctgtgccttacgagaagagtgaaaactgttcctcggcgccgatatttgttaggcaatccaacttcaagcttccttctgatcctttagtacctatcatcatgattggacctggcacagggttggcacctttcaggggcttcttacaggaaaggttggcattgaaaaatgatggggtggaacttggtcattctattctcttctttggatgcagaaaccgcaaaatggacttcatttacgaggatgagttgaacaattttgtcaaaacaggcgccctttctgagttgattgtagccttctcccgtgagggtccaactaaacaatatgtgcaacataaaatgactgagaaagcaacggaactttggaatatcatctcccaaggcggatatgtatacgtgtgtggagatgctaagggcatggctagagatgttcacagagttcttcatactattgctcaagagcagggaggtatggatagctccaaaacagaaagcttcatcaagagtttgcaaatggaagggagatacctaagagatgtatggtgaggatccggctgctaacaaagcccgaaaggaagctgagttggctgctgccaccgctgagcaataactagcataaccccttggggcctctaaacgggtcttgaggggttttttgctgaaaggaggaactatatccggccggatatccacaggacgggtgtggtcgccatgatcgcgtagtcgatagtggctccaagtagcgaagcgagcaggactgggcggcggccaaagcggtcggacagtgctccgagaacgggtgcgcatagaaattgcatcaacgcatatagcgctagcagcacgccatagtgactggcgatgctgtcggaatggacgatatcccgcaagaggcccggcagtaccggcataaccaagcctatgcctacagcatccagggtgacggtgccgaggatgacgatgagcgcattgttagatttcatacacggtgcctgactgcgttagcaatttaactgtgataaactaccgcattaaagcttatcgatgataagctgtcaaacatgagaattcttgaagacgaaagggcctcgtgatacgcctatttttataggttaatgtcatgcatgagacaataaccctgataaatgcttcaataatattgaaaaaggaagagtatgagtattcaacatttccgtgtcgcccttattcccttttttgcggcattttgccttcctgtttttgctcacccagaaacgctggtgaaagtaaaagatgctgaagatcagttgggtgcacgagtgggttacatcgaactggatctcaacagcggtaagatccttgagagttttcgccccgaagaacgttttccaatgatgagcacttttaaagttctgctatgtggcgcggtattatcccgtgttgacgccgggcaagagcaactcggtcgccgcatacactattctcagaatgacttggttgacgcgtcaccagtcacagaaaagcatcttacggatggcatgacagtaagagaattatgcagtgctgccataaccatgagtgataacactgcggccaacttacttctgacaacgatcggaggaccgaaggagctaaccgcttttttgcacaacatgggggatcatgtaactcgccttgatcgttgggaaccggagctgaatgaagccataccaaacgacgagcgtgacaccacgatgcctgcagcaatggcaacaacgttgcgcaaactattaactggcgaactacttactctagcttcccggcaacaattaatagactggatggaggcggataaagttgcaggaccacttctgcgctcggcccttccggctggctggtttattgctgataaatctggagccggtgagcgtgggtctcgcggtatcattgcagcactggggccagatggtaagccctcccgtatcgtagttatctacacgacggggagtcaggcaactatggatgaacgaaatagacagatcgctgagataggtgcctcactgattaagcattggtaactgtcagaccaagtttactcatatatactttagattgatttaaaacttcatttttaatttaaaaggatctaggtgaagatcctttttgataatctcatgcatgaccaaaatcccttaacgtgagttttcgttccactgagcgtcagaccccgtagaaaagatcaaaggatcttcttgagatcctttttttctgcgcgtaatctgctgcttgcaaacaaaaaaaccaccgctaccagcggtggtttgtttgccggatcaagagctaccaactctttttccgaaggtaactggcttcagcagagcgcagataccaaatactgtccttctagtgtagccgtagttaggccaccacttcaagaactctgtagcaccgcctacatacctcgctctgctaatcctgttaccagtggctgctgccagtggcgataagtcgtgtcttaccgggttggactcaagacgatagttaccggataaggcgcagcggtcgggctgaacggggggttcgtgcacacagcccagcttggagcgaacgacctacaccgaactgagatacctacagcgtgagctatgagaaagcgccacgcttcccgaagggagaaaggcggacaggtatccggtaagcggcagggtcggaacaggagagcgcacgagggagcttccagggggaaacgcctggtatctttatagtcctgtcgggtttcgccacctctgacttgagcgtcgatttttgtgatgctcgtcaggggggcggagcctatggaaaaacgccagcaacgcggcctttttacggttcctggccttttgctggccttttgctcacatgttctttcctgcgttatcccctgattctgtggataaccgtattaccgcctttgagtgagctgataccgctcgccgcagccgaacgaccgagcgcagcgagtcagtgagcgaggaagcggaagagcgcctgatgcggtattttctccttacgcatctgtgcggtatttcacaccgcatatatggtgcactctcagtacaatctgctctgatgccgcatagttaagccagtatacactccgctatcgctacgtgactgggtcatggctgcgccccgacacccgccaacacccgctgacgcgccctgacgggcttgtctgctcccggcatccgcttacagacaagctgtgaccgtctccgggagctgcatgtgtcagaggttttcaccgtcatcaccgaaacgcgcgaggcagctggcacgacaggtttcccgactgggttggtgcgttttatcatgcctggcgggtaggtcggataaggcgttcacgccgcatccgacaaccacgcagcgttacctgatgtgacgccgacaattctcatcatcgctacaacatgacctcgctatttacatcgcgatactcttttggcgtcgtgtcatatgcttttttaaaaacagagtagaaatattgcagcgatggataaccgcacatttgcgatatctcattgatcgacaaggtggttgaaatcagcagactgcgcgctttctccagcttctcggcatgaatcatggcatggatggtttcacccacctcttctttaaaacgcttctcaagattggagcgcgagatcccgaccgcatccagtacctgatccactttaatccctttacaggcgtgattacgaatgtaatgcatggcctgaataacggcgggatcggtcagcgagcgataatctgttgagcgccgttcaatgacgcgaactggtgggaccaaaattcgctgtagcggcatttcttctttatctaataatcgatgcaacagttttgccgcctgatagcccatttgccgcgcgccctgagcgaccgaagaaagggcgacacgcgacagatagcgggtcagttcttcgttatcgatgccaatcacgcataatttttccggtacgggaatatgtagatgttcacatacttgcagaatatgccgcgctcgggcgtcagtaacggcaataatcccggtttgcggtggtagcgtttgtagccagtctgccagccgattttgcgcgtgttgccagttctctggcgcggtttctaacccctgataaaccactccgcgatacttttcttcggcgacaagctgacgaaatgcatattcgcgctcagtggcccaacgtttgccgcttgattccggaagaccataaaaagcaaagcggttaacgcctttctcttttaaatgcaaaaatgcgctttcaaccagcgcatagttatcggtggcaatgtaatgaacgggtgggtaactttctgcaaggtgatacgagccgccaaccccaacaatggggacgtcgacatcagccagcgcttgctcgatctgtttgtcgtcgaagtcggcaatgacgccatctcctaaccagtccttgattttatcaatgcgggcgcggaaatcttcttcaatgaaaatatcccattccgattgtgacgcctgtaaatattcccctacgccttctactacctgccggtcataggctttattggcattgaacagtaatgtgatgcggtgacgtttagtaaacatggttcttttcctgctgaatcatgctaagtaacaatcaccgcgataaacgtaaccaatttttagcaactaaacaggggaaaacaattacagatttttatctttcgattacgatttttggtttatttcttgatttatgaccgagatcttacttttgttgcgcaattgtacttattgcatttttctcttcgaggaatt

SEQ ID NO: 12 - DNA, 6779 bp, pGT1681
gagtgtatactggcttactatgttggcactgatgagggtgtcagtgaagtgcttcatgtggcaggagaaaaaaggctgcaccggtgcgtcagcagaatatgtgatacaggatatattccgcttcctcgctcactgactcgctacgctcggtcgttcgactgcggcgagcggaaatggcttacgaacggggcggagatttcctggaagatgccaggaagatacttaacagggaagtgagagggccgcggcaaagccgtttttccataggctccgcccccctgacaagcatcacgaaatctgacgctcaaatcagtggtggcgaaacccgacaggactataaagataccaggcgtttccccctggcggctccctcgtgcgctctcctgttcctgcctttcggtttaccggtgtcattccgctgttatggccgcgtttgtctcattccacgcctgacactcagttccgggtaggcagttcgctccaagctggactgtatgcacgaaccccccgttcagtccgaccgctgcgccttatccggtaactatcgtcttgagtccaacccggaaagacatgcaaaagcaccactggcagcagccactggtaattgatttagaggagttagtcttgaagtcatgcgccggttaaggctaaactgaaaggacaagttttggtgactgcgctcctccaagccagttacctcggttcaaagagttggtagctcagagaaccttcgaaaaaccgccctgcaaggcggttttttcgttttcagagcaagagattacgcgcagaccaaaacgatctcaagaagatcatcttattaatcagataaaatatttctagatttcagtgcaatttatctcttcaaatgtagcacctgaagtcagccccatacgatataagttgtaattctcatgtttgacagcttatcatcgataagctttaatgcggtagtttatcacagttaaattgctaacgcagtcaggaaccttgcaatgcattatccgtttataaggacagcccgaatgacggtctgcgcaaaaaaacacgttcatctcactcgcgatgctgcggagcagttactggctgatattgatcgacgccttgatcagttattgcccgtggagggagaacgggatgttgtgggtgccgcgatgcgtgaaggtgcgctggcaccgggaaaacgtattcgccccatgttgctgttgctgaccgcccgcgatctgggttgcgctgtcagccatgacggattactggatttggcctgtgcggtggaaatggtccacgcggcttcgctgatccttgacgatatgccctgcatggacgatgcgaagctgcggcgcggacgccctaccattcattctcattacggagagcatgtggcaatactggcggcggttgccttgctgagtaaagcctttggcgtaattgccgatgcagatggcctcacgccgctggcaaaaaatcgggcggtttctgaactgtcaaacgccatcggcatgcaaggattggttcagggtcagttcaaggatctgtctgaaggggataagccgcgcagcgctgaagctattttgatgacgaatcactttaaaaccagcacgctgttttgtgcctccatgcagatggcctcgattgttgcgaatgcctccagcgaagcgcgtgattgcctgcatcgtttttcacttgatcttggtcaggcatttcaactgctggacgatttgaccgatggcatgaccgacaccggtaaggatagcaatcaggacgccggtaaatcgacgctggtcaatctgttaggcccgagggcggttgaagaacgtctgagacaacatcttcagcttgccagtgagcatctctctgcggcctgccaacacgggcacgccactcaacattttattcaggcctggtttgacaaaaaactcgctgccgtcagttaataccgcccttttgggttcaagcagtacataacgatggaaccacattacaggagtagtgatgaatgaaggacgagcgccttgttcagcgtaagaacgatcatctggatatcgttctcgacccccgtcgcgccgtaactcaggctagcgcaggttttgagcgctggcgctttacccactgcgccctgccagagctgaattttagcgacatcacgctggaaaccaccttcctgaatcggcagctacaggctccgctgctgatcagctccatgaccggcggcgttgagcgctcgcgccatatcaaccgccacctcgccgaggcggcgcaggtgctaaaaattgcgatgggggtgggctcccagcgcgtcgccattgagagcgacgcgggcttagggctggataaaaccctgcggcagctggctccggacgtgccgctgctggcgaacctcggcgcggcgcagctgaccggcagaaaaggtattgattacgcccgacgggccgtggagatgatcgaggcggatgcgctgattgtgcacctaaacccgctgcaggaggcgctacagcccggcggcgatcgcgactggcgcggacggctggcggctattgaaactctggtccgcgagctgcccgttccgctggtggtgaaagaggtgggagccggtatctcccgaaccgtggccgggcagctgatcgatgccggcgttaccgtgattgacgtcgcgggcgcgggcggcaccagctgggccgccgttgaaggcgagcgggcggccaccgagcagcagcgcagcgtggccaacgtctttgccgactgggggatccccaccgctgaggcgctggttgacattgccgaggcctggccgcagatgccccttattgcctcgggcgggattaaaaacggcgtcgacgcggcgaaagcgctgcggctcggcgcgtgcatggtagggcaggccgccgccgtgctcggcagcgcaggcgtctccacggagaaggtgatcgatcacttcaacgtgattattgagcagctgcgggtggcctgcttctgcaccggcagccgcagcctgagcgatctaaagcaggctgatatccgctatgtgcgtgatacgccataaggaggtacaaccatgacagcggcagagacacggccggaccagctgccgcaagaagaaaggttcgtaagtcgcctaaatgccgattatcaccctgccgtgtggaaggacgactttattgatagtttaaccagcccgaacagccatgcaacctccaaatcgtctgttgatgaaactatcaataaacgtatccagaccttggtgaaagaaatacaatgcatgtttcagagcatgggcgatggtgaaacgaatccttctgcttacgataccgcgtgggtggcaagaataccgtcgatcgacggcagtggcgcaccgcagtttccccagacacttcagtggattttaaacaatcagctgccggatggtagctggggtgaagaatgcatctttttggcatatgatcgagtgctgaatacgttagcttgcttgcttacgctcaagatctggaacaaaggcgatattcaagttcagaaaggcgtcgagttcgtacgtaaacatatggaggagatgaaagatgaggccgacaatcatcggccttccgggttcgaggtggtatttccggccatgttagatgaagctaagagccttggcctggacctgccataccatctgccttttattagccagatccaccaaaaacggcaaaagaaattacagaaaattccgttaaatgttttacataaccatcagacagcgcttttatactctctcgaggggctgcaggatgttgtcgattggcaggaaattactaatcttcaatcgcgtgatggaagttttctgagcagtccggcttccaccgcttgtgtcttcatgcatacacaaaacaaacgctgtttgcatttcctgaactttgtgttatctaagttcggtgactatgtaccttgtcactacccgttggatctctttgaacgcctgtgggcggttgacacggtagaacgtctcggcatcgataggtattttaaaaaagaaattaaagaaagccttgattatgtgtaccgttactgggacgcagaacgaggagtgggctgggcgcgatgtaacccgattccagatgtcgatgacaccgcaatggggctgcgaatcctacgcctgcatggctataacgtcagctccgacgtcctggagaatttccgggatgaaaagggcgacttcttttgcttcgcgggccagactcagataggggttaccgataatctgaatctgtaccgttgtagtcaggtgtgctttcctggtgaaaaaattatggaagaagcgaagacgtttacgactaaccacctgcaaaacgccctggccaaaaataacgcattcgataagtgggctgtcaagaaggatctgccgggcgaagtagaatacgccattaagtatccctggcatcgctccatgccgcgtctggaagcccgttcctatatcgagcagtttggttcaaatgacgtctggctcggtaaaacagtatacaaaatgctgtatgttagcaacgagaaatatcttgagctggccaaactggatttcaatatggttcaagctttgcaccaaaaggaaacgcaacacattgtgtcatggtggcgcgagtctggctttaatgatctgacgtttactcgtcagcgtccggtagaaatctatttctccgtggcggtgagtatgttcgaaccagagttcgccgcttgtcgcattgcctacgcaaaaacctcatgcctcgcggtgatcctggacgatctgtatgatacgcatggtagtctggatgacctcaaattgtttagcgaggcggtccgccgttgggatattagtgttcttgacagcgtgcgcgataaccaactgaaggtgtgttttctcggactgttcaacacagtgaacggtttcggcaaagatgggctgaaagaacagggccgcgatgtcttgggttatttgcgcaaggtgtgggaaggtttgctagcgtcctacacgaaagaggcggaatggagcgcagcaaagtatgtgccaacctttaatgaatatgtcgagaatgcaaaagtttcaattgcgctcgccaccgtagttctgaattcaatcttctttaccggcgagctgctgccagattacattctccagcaggtagacctgcgctcgaaattcttacatctggtgagtctcaccggccgtttgataaacgataccaaaacataccaggccgaacgtaaccgcggggagctggtttcttcggtccaatgttacatgcgcgagaacccggagtgtactgaagaggaagctctcagccacgtctacggcataattgacaacgcactgaaggaactgaactgggagctagcaaaccctgcgtccaacgcgcccttatgcgtgcgccgtctgttgtttaataccgctcgtgtcatgcagcttttttacatgtatcgtgacggttttggaatttcggataaagaaatgaaagatcacgtgtcccgtaccttatttgacccggtagcatgaggatccggctgctaacaaagcccgttctgtttaagaacgggattttttgctgaaaggaggaactatatccggccggatatcccgcgcgcttgtttcggcgtgggtatggtggcaggccccgtggccgggggactgttgggcgccatctccttggggtcgaatttgctttcgaatttctgccattcatccgcttattatcacttattcaggcgtagcaccaggcgtttaagggcaccaataactgccttaaaaaaattacgccccgccctgccactcatcgcagtactgttgtaattcattaagcattctgccgacatggaagccatcacagacggcatgatgaacctgaatcgccagcggcatcagcaccttgtcgccttgcgtataatatttgcccatggtgaaaacgggggcgaagaagttgtccatattggccacgtttaaatcaaaactggtgaaactcacccagggattggctgagacgaaaaacatattctcaataaaccctttagggaaataggccaggttttcaccgtaacacgccacatcttgcgaatatatgtgtagaaactgccggaaatcgtcgtggtattcactccagagcgatgaaaacgtttcagtttgctcatggaaaacggtgtaacaagggtgaacactatcccatatcaccagctcaccgtctttcattgccatacggaattccggatgagcattcatcaggcgggcaagaatgtgaataaaggccggataaaacttgtgcttatttttctttacggtctttaaaaaggccgtaatatccagctgaacggtctggttataggtacattgagcaactgactgaaatgcctcaaaatgttctttacgatgccattgggatatatcaacggtggtatatccagtgatttttttctccattttagcttccttagctcctgaaaatctcgataactcaaaaaatacgcccggtagtgatcttatttcattatggtgaaagttggaacctcttacgtgccgatcaacgtctcattttcgccaaaagttggcccagggcttcccggtatcaacagggacaccaggatttatttattctgcgaagtgatcttccgtcacaggtatttattcggcgcaaagtgcgtcgggtgatgctgccaacttactgatttagtgtatgatggtgtttttgaggtgctccagtggcttctgtttctatcagctgtccctcctgttcagctactgacggggtggtgcgtaacggcaaaagcaccgccggacatcagcgctagcg

SEQ ID NO: 13 - DNA, 708 bp, Curcuma wenyujin
atggcagccgtagccgacgatgccagcatggatgctgttcagcgccgtcttatgtttgaagatgaatgtattctcgttgacgaaaacgacgttgtgattggacatgagtcgaaatataattgccatcttgtcgaaaagattgagtcgttgaacctcttgcaccgtgcgttttcagtgtttctgtttaatagcaaatatgaattacttttacagcaacgcagtgaaaccaaggtgaccttccccctggtctggacaaacacctgctgcagccaccccttgtaccgcgagtctgagttaattcaagaaaactacctgggtgtgcgcaatgccgcgcagcgtaaactcctggatgaactgggcattcctgcggaggacattccagtggatgagtttatcccgctgggccgtatgctgtacaaggcgccatccgacggtaaatggggcgagcatgaggtagattatttgctgtttatcgtgcgcgatgtgaaactgctgccgaatccggatgaagtggcggatgtaaagtatgtcaatcgtgatcagctgaaagagctgctgcgcaaggcggatgccggagaggaaggtgtgaaactgtcaccttggttccgcttggtcgtggacaactttctgatggaatggtgggcgcgtgtggaacagggtaccctgctggaggcagccgatatggaaacaatccataagctggtctaa

SEQ ID NO: 14 - protein, 235 aa, Curcuma wenyujin
MAAVADDASMDAVQRRLMFEDECILVDENDVVIGHESKYNCHLVEKIESLNLLHRAFSVFLFNSKYELLLQQRSETKVTFPLVWTNTCCSHPLYRESELIQENYLGVRNAAQRKLLDELGIPAEDIPVDEFIPLGRMLYKAPSDGKWGEHEVDYLLFIVRDVKLLPNPDEVADVKYVNRDQLKELLRKADAGEEGVKLSPWFRLVVDNFLMEWWARVEQGTLLEAADMETIHKLV

SEQ ID NO: 15 - DNA, 2394 bp, Abies grandis
atgagcgctgaaaagaatgattcgctttcgtcgtcaactctggtaaagcgagagttcccgccgggattctggaaagacgacttgatcgactcgcttaccagcagtcacaaagtggccgctagtgacgaaaagcgcatagaaactcttatcagtgaaattaagaatatgttccgttgtatgggatatggagaaaccaatcccagtgcatacgacacggcatgggtggctcgaattccagcagtagatggttccgataatcctcactttccagaaacagttgaatggattttacaaaaccagctaaaagatgggtcatggggtgaaggtttctacttcctcgcttatgaccggattctagccactttagcttgtatcattacactcacgctatggcgcacaggggaaacccaggtacagaagggtattgagttcttccggacccaagcaggcaagatggaagatgaggcagattctcaccgtccgtccgggttcgagatagtcttccccgctatgttgaaagaggctaagattctgggcttggacctgccatacgacctccctttcctcaagcagattatcgagaagagagaagctaaactgaaacgtatacctaccgatgtcttatatgccttgcctacgacccttttgtactcgttggagggactccaagaaatcgtggactggcaaaagattatgaaattgcaatccaaagacggctcattcttgtcaagccccgcgtcgactgctgcagtgtttatgcgtaccggcaacaagaaatgtttagacttcttaaatttcgtactgaagaagttcggtaaccatgtgccgtgccattacccgttggatcttttcgagcggttgtgggctgtcgacactgttgagaggctcggaatagaccgtcatttcaaggaggagataaaagaggctctcgactacgtatattctcattgggatgaacgcggcataggttgggcgagagaaaatccagtcccggacatagacgacaccgcaatgggcctcagaatcctgcgcctacacgggtacaatgtgtcgtctgatgtgctgaaaactttccgcgacgaaaatggggaattcttctgtttcctaggtcagacccagcgaggagtgaccgatatgttgaacgtcaatcggtgcagtcatgtgtcctttccaggcgagactatcatggaagaagccaagctctgtactgaacggtacctccgaaacgcgctcgagaatgtagatgcatttgacaaatgggcattcaagaagaacattcgaggagaggttgagtacgccttaaagtatccgtggcataagtcgatgcctaggctagaggcccggtcgtacatagagaactatggtccggatgatgtctggttgggcaagactgtgtacatgatgccctatattagcaacgaaaagtatctggagttagccaaactagactttaataaggttcaaagcatccaccaaacggagctgcaagatcttagacgttggtggaagagcagtgggttcaccgatctcaatttcacgcgagaacgtgtcactgagatatattttagccctgcctcgttcatcttcgaacccgaattctctaaatgtagggaggtttacacaaagacaagtaactttactgttatactggacgacctatacgacgcgcacgggagtcttgacgacctgaagctgttcactgagagtgtgaaacgctgggacctgagtctcgtcgaccaaatgccgcagcagatgaagatctgctttgtgggcttctataatacttttaacgacattgcgaaggagggcagggaacgccaaggacgtgacgtactgggatacattcagaacgtctggaaagtacaactcgaggcatatacaaaggaggctgaatggtcggaggctaagtatgttccgtctttcaacgaatacatcgaaaacgcatcggtgtcaatagccttgggcacggtagtcctaatctcggctcttttcactggggaagtcttgaccgatgaggttctctcaaagattgaccgggaatcgagatttcttcaattgatgggtctcaccggtcgattagtcaacgatacgaagacgtatcaagcagagaggggtcagggtgaagtagctagcgctattcaatgttacatgaaggaccatcccaagatatccgaggaggaggctcttcagcatgtatactcagtcatggagaacgctctcgaagagttaaacagagaatttgtcaacaataagatccctgacatctacaagaggctggtgttcgaaaccgctcgcatcatgcagctattctacatgcaaggcgatggtctcaccctttcccatgacatggaaataaaggagcacgttaagaactgcctattccagccagtcgcc

SEQ ID NO: 16 - protein, 798 aa, Abies grandis
MSAEKNDSLSSSTLVKREFPPGFWKDDLIDSLTSSHKVAASDEKRIETLISEIKNMFRCMGYGETNPSAYDTAWVARIPAVDGSDNPHFPETVEWILQNQLKDGSWGEGFYFLAYDRILATLACIITLTLWRTGETQVQKGIEFFRTQAGKMEDEADSHRPSGFEIVFPAMLKEAKILGLDLPYDLPFLKQIIEKREAKLKRIPTDVLYALPTTLLYSLEGLQEIVDWQKIMKLQSKDGSFLSSPASTAAVFMRTGNKKCLDFLNFVLKKFGNHVPCHYPLDLFERLWAVDTVERLGIDRHFKEEIKEALDYVYSHWDERGIGWARENPVPDIDDTAMGLRILRLHGYNVSSDVLKTFRDENGEFFCFLGQTQRGVTDMLNVNRCSHVSFPGETIMEEAKLCTERYLRNALENVDAFDKWAFKKNIRGEVEYALKYPWHKSMPRLEARSYIENYGPDDVWLGKTVYMMPYISNEKYLELAKLDFNKVQSIHQTELQDLRRWWKSSGFTDLNFTRERVTEIYFSPASFIFEPEFSKCREVYTKTSNFTVILDDLYDAHGSLDDLKLFTESVKRWDLSLVDQMPQQMKICFVGFYNTFNDIAKEGRERQGRDVLGYIQNVWKVQLEAYTKEAEWSEAKYVPSFNEYIENASVSIALGTVVLISALFTGEVLTDEVLSKIDRESRFLQLMGLTGRLVNDTKTYQAERGQGEVASAIQCYMKDHPKISEEEALQHVYSVMENALEELNREFVNNKIPDIYKRLVFETARIMQLFYMQGDGLTLSHDMEIKEHVKNCLFQPVA

SEQ ID NO: 17 - DNA, 2358 bp, Pinus contorta
atggccaagcgcgaagagattccgcccggcgtatggaaggacgacatctctgatagcattatgagttcacataagccagaagccgatgaaaaacgtgtcgaaatcctgattgcggagattaaatcaatgtttcgcgggatgggagatggcgagaccactccgtcagcctatgatacggcgtgggtggccaagattcctgcgctggatggttcggaccaccctcactttccgcaaaccctgcagtggattctccagaaccaattacaagacggaagctggggcgaaggtacctatttctccacgtatgaccggctcctcgcgaccttagcctgtatcattacgctcacagtctggcgcactggccagacccaggtgcgacagggcattgagtttttccgcaaacatgcagggactatggaggatgaggcggataaccatcaaccgataggatttgaattcgtttttcccgcgatgattaatgaagccaaaagtctgtgtctggatctgccgtacgacacccctttcatcaaacaaattatcgaaaagcgcgaagcgaaattgaaaatgattccgacggatacgctgtacacggtgcctactacgttcctctactacttagaagggctacaagagatcatcgactgccaaaaaataattaagttgcaaagcaaagatggttcatttttgagtagtcccgcctcgaccgcggcggtttttatgtgcaccggcaataccaagtgtctcgagtttcttaactttgtgctgattaagttcggtaatcacgtgccgtgccaatacccgctggatttatttgaaagattatgggcagttgatatcgtggaacgcctgggcattgaccgccatttcaaaaaagagattaaggatgcattagattacgtctatagtcattgggacgaacgtgggattcgatgggcacgagaaaacccagtcgcgtatatcgatgttatggccacaggcattcgtatactgaggctgcatcgttacaacgtgagctctgacatcctgaaaacctttcgagatgaaaacggagagttttatcgcttcccaggccaatccgagcggggtgttaccgatatgctgaacttgaaccgctgcagccacgtggcatttccaggtgaaactgtcatggaggaagcaaagttatgtacagaaagatacctgtggaacgcgttggagaatgtcaatcccctggacaagtggggtctgaaggagaatatccgcggtgaagttgagtatgcgttgaaatatccgtggcttcgccgtttgccccgtttggaaacgcgtaactacatcgagcattacggggcaaacgatgtgtggctgggcaagatgatgcacatgatgccctacatcaatgatcgcaaatacctggagctcgctaaattggactttaataatgtacagagcatacatcaaaaggaactgcgcgaattgcgtcgttggtggaagtcatctggttttgccgaacttaactttctgccagaccgagtcgccgagatcttcttctccatcgcaagttcaatgttcgaaccggaactggctacctgccgcgcggtatacactaaatccacactgtgcactgtcattctggacggcttctatgacgttcacgggtcggccgaagacattatgttattcaatgaagcggtcaaacgctgggatcactctctgctcgatcgtatggccgaacatatcaaaacgtgttttcttgctctgtacaacgttgttaacgaaattgcggaagagggtcgtaagcgtcagggccatgacgtgctgccgtatattcgtaatttatgggaaatccagcttgaatctttcacgaaagaagcagaatggtcgagagctgaacatgtgccgtccttccatgaatacatagaggccgctgccatatcatcagcactgccaactctcgttctgattggcgttattttcactggagaggttctcacagatcacatactctcccaaattgattaccgatccaaatttgcatatctcatgagcttgacagggcgtttggcgaacgataccaaaacttaccaggtggagagaggtcaaggagaggtggcttctgccatacagtgttacatgaaggaaaatcccgaattgtcagaggaagaagctctcgaatatatttataggctcatggaaaacgccctcgcagatttcaagtgtgaatttctgaataccaaagacgtgccggagtattgcagaagactagtttttgacaatgcgagatcaatgcagctgatttacatggaaggagacggtttcaaactttcacatgaaacggaaattaaacagcatgtcaaaaagatcctgttcgaaccagttgcc

SEQ ID NO: 18 - protein, 786 aa, Pinus contorta
MAKREEIPPGVWKDDISDSIMSSHKPEADEKRVEILIAEIKSMFRGMGDGETTPSAYDTAWVAKIPALDGSDHPHFPQTLQWILQNQLQDGSWGEGTYFSTYDRLLATLACIITLTVWRTGQTQVRQGIEFFRKHAGTMEDEADNHQPIGFEFVFPAMINEAKSLCLDLPYDTPFIKQIIEKREAKLKMIPTDTLYTVPTTFLYYLEGLQEIIDCQKIIKLQSKDGSFLSSPASTAAVFMCTGNTKCLEFLNFVLIKFGNHVPCQYPLDLFERLWAVDIVERLGIDRHFKKEIKDALDYVYSHWDERGIRWARENPVAYIDVMATGIRILRLHRYNVSSDILKTFRDENGEFYRFPGQSERGVTDMLNLNRCSHVAFPGETVMEEAKLCTERYLWNALENVNPLDKWGLKENIRGEVEYALKYPWLRRLPRLETRNYIEHYGANDVWLGKMMHMMPYINDRKYLELAKLDFNNVQSIHQKELRELRRWWKSSGFAELNFLPDRVAEIFFSIASSMFEPELATCRAVYTKSTLCTVILDGFYDVHGSAEDIMLFNEAVKRWDHSLLDRMAEHIKTCFLALYNVVNEIAEEGRKRQGHDVLPYIRNLWEIQLESFTKEAEWSRAEHVPSFHEYIEAAAISSALPTLVLIGVIFTGEVLTDHILSQIDYRSKFAYLMSLTGRLANDTKTYQVERGQGEVASAIQCYMKENPELSEEEALEYIYRLMENALADFKCEFLNTKDVPEYCRRLVFDNARSMQLIYMEGDGFKLSHETEIKQHVKKILFEPVA